European Patent Specification EP 3 911 180 B1, published May 21, 2025. Title: Paenibacillus wynnii beta-galactosidase for the production of lactose-depleted dairy products. Applicant: Universität Hohenheim. The sequence listing filed with the application follows.

SEQUENCE LISTING (2 sequences)

SEQ ID NO: 1 - protein, 1042 aa, Paenibacillus wynnii
MRKKLVYSPPTNGYPEWNNNPECFQINRMDAHATWIPFNTTEDALLGDPQSSPNYLSLNGMWKFAYAETPDQRIRNFFEKNYDCSSWAELNVPSHWQMHGYDYPQYTNVRYPWSEREPELKPPFAPTQYNPVGSYVRTFSVPEDWSGKPVFISFQGVESAFYVWLNGELVGYSEDTFTPAEFDLTPYLIPGDNKLAVEVYRWCDASWLEDQDFWRLSGIFRDVYLYTTPEAHIYDFFVRTELDEQYRHAELQLDVKLMDYFERTAEAVIVHAQLYDHDQNAIFDQPLSQTVYFNSASTQTLQFSSSIIDPLKWSAEHPNLYTLVLSLHHVDGELMEAVSCRVGFRTFELKDGLMKINGKRIVFKGVNRHEFSCDTGRSIDVDDMVRDILLMKAHNINAVRTSHYPNQTIWYDLCDQYGLYVIDETNLETHGSWSYGQTDLGGNTVPGSRPEWRANVLDRCNSMLQRDKNHPSIVIWSLGNESFGGDNFVAMHDFLKKEDPSRLVHYEGLFHYRESDVASDIESTMYISPADVEQYALNDPKKPYILCEYSHAMGNSCGGLHLYWEVFEKYDILQGAFIWDWIDQAIRLKQADGSMHMAYGGDFGESPHDGNFCGNGLIFADRSVSPKLYEVKKCYQNVKFEAVDLERGIYRVTNQNLFTDLAEYALAWEVSCNGNPVLKGTVDLAVPAGESAEISVPVVDEPNLQSEGEHVLTFSLQLKKSTLWADAGHEVAWEQFLLPTPQFMAGQDQDSVLTSDRGVIVEEQAGRLTVQAADVSLQFSTSSGYLISMQNKGKELLLEPVRPNFWRAVTDNDLGNKHHERCAVWNTAGAGCTLASFESHKNVDGVTVRAKYTVPTVPISSLILEYRIQENGSIEVFEELSPGMGLPEIPEIGLMFIVEDRLDTVSWYGRGPHENYWDRKTGARLGYFSGSVQDQFVPYIRPQECGNKTDVRFASITGGINGSGFRVDGDPVLELNALPWTPAELEANDHIYKLPASNKTVVRVNYKQMGVGGDNSWGATTHPEFTLPADQTYGFRFTIRMV

SEQ ID NO: 2 - DNA, 3129 bp, Paenibacillus wynnii
atgcgtaaaaaacttgtctattcaccccctaccaacgggtacccggaatggaataataatcccgaatgttttcagatcaaccgaatggatgcccatgctacatggataccttttaatacaacagaggatgccttgcttggagatccacaatcctcgcccaactatttgtctttgaatgggatgtggaaattcgcctatgcagagactccggatcaacgcatacgtaacttttttgaaaaaaactatgattgcagttcttgggctgaactgaacgttccctctcattggcagatgcatggatatgactaccctcagtatacgaatgtacggtatccctggagtgaacgtgagccggagctcaaaccgccttttgctcccacccaatataatccggttgggtcttatgtacgaaccttctctgtaccggaggactggagcgggaagcctgttttcatcagctttcaaggtgtggagtctgccttctatgtttggctcaatggagagttggtcggatacagcgaggataccttcacccctgcggaatttgacttaactccttatctaatcccgggagacaataagcttgccgttgaagtgtatcgttggtgtgacgccagttggctggaggatcaggatttctggagacttagcggcatatttagagatgtctatctatatacaacaccggaagcccatatttatgatttctttgttcgaacagaactggatgagcagtaccggcatgctgaattgcagctggatgtgaagcttatggattattttgaaagaaccgctgaggcagttattgtgcatgcgcagctttatgatcacgatcagaacgctatctttgatcagccgctttcacagacagtctacttcaatagcgcttctacccagacgctccaattctcttcttctattattgacccgttaaaatggagtgcggaacatccgaatctatatacgttagtgttgtctttacatcatgtggatggagagctcatggaagccgttagctgccgtgttggctttcgtacattcgagctaaaggacggtttaatgaagattaatggaaaacggatcgtctttaagggcgtgaaccgccatgaattctcatgcgataccggcagatcaattgatgtcgatgatatggtacgggacattctactgatgaaagcacacaacatcaatgccgttcggacttcgcattatccgaatcagaccatatggtatgacctttgtgaccaatatgggctgtatgtaattgatgagaccaatctggagacacatggttcgtggagctatggacagacagacttaggcggaaatacggtacccggcagtagacctgaatggcgcgcgaatgtactggatcggtgtaattcaatgctccaaagggacaaaaaccacccttccatcgtcatctggtcactcggtaacgagtcctttggcggtgataactttgtggctatgcatgattttcttaagaaagaagacccctcccggcttgtccattatgaaggcctctttcactatcgcgagagcgatgttgcctcggacattgagagcaccatgtacattagtccggccgatgtggaacagtatgcgcttaatgatccaaagaagccttatattctatgcgagtatagccatgcaatgggcaactcctgcgggggattgcatctatactgggaagtttttgagaaatatgatattttacagggtgcctttatctgggactggattgatcaagcgattcgacttaagcaagccgacggatccatgcatatggcctacggcggagacttcggggaatcccctcatgacggcaacttctgcggaaatggcttgattttcgctgaccgttcagtatctcctaagctgtatgaggtcaagaaatgctaccagaatgttaaatttgaggctgtcgatttagagcgaggcatttatcgggtaaccaatcagaatctatttacggatttggcggagtacgcactggcttgggaagtaagctgtaacggcaatcctgtgcttaagggtactgttgatctggctgtccctgcaggagaatcggcagaaatttcggttcccgtggtcgatgaacctaacctgcaatccgagggcgagcatgtcctcacgtttagcctgcaattgaagaaatccaccctttgggcagacgcaggccatgaagtggcatgggaacaattcctgctgcctacacctcagtttatggcgggtcaggatcaagactctgttttgacatcagatcgtggtgtgattgtggaggaacaagcagggcgtttaactgttcaggcggcggatgtctcccttcaattcagtacttcaagcggttatctgatctctatgcaaaataaaggcaaggaactgctgctcgaacctgttcgtccgaatttctggcgtgcagttacggataacgatctagggaacaaacaccatgagcgttgcgcggtttggaatacagcgggagctggctgtacactagcttcctttgaatcgcataagaatgtagatggcgtaactgttcgtgctaagtacaccgtacccaccgtacccatttcttcactgatattggaatatagaatccaagaaaatggctccattgaagtctttgaagagctatcaccgggcatgggcttgccggagattcctgaaattggcctcatgtttatcgttgaagatcgactcgacaccgtttcatggtatggccgcggaccgcatgagaattactgggaccggaagacaggcgccagacttggatatttttcgggaagtgtccaggatcagttcgttccgtatataaggcctcaagaatgcggaaacaaaacggatgtgcgttttgccagtatcactgggggtataaacggctcaggattccgtgtggatggcgatcctgtactggaactaaatgccttgccttggacacccgctgagttggaagcgaatgatcacatatataagctgccagccagtaataaaaccgttgtgcgtgtgaactacaagcaaatgggtgtaggtggagacaacagctggggcgcgacgacacatcctgaattcactttgccggcggatcaaacttatgggtttcggtttacgattcggatggtgtaa